European Patent Specification EP 3 349 783 B1, published January 17, 2024. Title: Compositions And Methods Relating To The Treatment Of Diseases. Applicant: Alfacyte Ltd. The sequence listing filed with the application follows.

SEQUENCE LISTING (5 sequences)

SEQ ID NO: 1 - protein, 166 aa, Homo sapiens
CDLPQTHSLGNRRALILLGQMGRISPFSCLKDRHDFRIPQEEFDGNQFQKAQAISVLHEMMQQTFNLFSTKNSSAAWDETLLEKFYIELFQQMNDLEACVIQEVGVEETPLMNEDSILAVKKYFQRITLYLIERKYSPCAWEVVRAEIMRSLSFSTNLQKRLRRKD

SEQ ID NO: 2 - protein, 507 aa, Homo sapiens
ATGTGTGATCTGCCGCAGACCCATAGCCTGGGTAATCGTCGTGCACTGATTCTGCTGGGTCAGATGGGTCGTATTAGCCCGTTTAGCTGTCTGAAAGATCGTCATGATTTTCGTATTCCGCAAGAGGAATTTGATGGCAACCAGTTTCAGAAAGCACAGGCAATTAGCGTTCTGCATGAAATGATGCAGCAGACCTTTAACCTGTTTAGCACCAAAAATAGCAGCGCAGCATGGGATGAAACCCTGCTGGAAAAATTCTATATCGAACTGTTTCAGCAGATGAACGATCTGGAAGCATGTGTTATTCAAGAAGTTGGCGTTGAAGAAACACCGCTGATGAATGAAGATAGCATTCTGGCAGTGAAAAAATACTTTCAGCGCATTACCCTGTATCTGATCGAACGTAAATATAGCCCGTGTGCATGGGAAGTTGTTCGTGCAGAAATTATGCGTAGCCTGAGCTTTAGCACCAATCTGCAAAAACGTCTGCGTCGCAAAGATTAATAA

SEQ ID NO: 3 - protein, 498 aa, Homo sapiens
TGYGAYYTNCCNCARACNCAYWSNYTNGGNAAYMGNMGNGCNYTNATHYTNYTNGGNCARATGGGNMGNATHWSNCCNTTYWSNTGYYTNAARGAYMGNCAYGAYTTYMGNATHCCNCARGARGARTTYGAYGGNAAYCARTTYCARAARGCNCARGCNATHWSNGTNYTNCAYGARATGATGCARCARACNTTYAAYYTNTTYWSNACNGARAAYWSNWSNGCNGCNTGGGARCARACNYTNYTNGARAARTTYWSNATHGARYTNTTYCARCARATGAAYGAYYTNGARGCNTGYGTNATHCARGARGTNGGNGTNGARGARACNCCNYTNATGAAYGARGAYWSNATHYTNGCNGTNMGNAARTAYTTYCARMGNATHACNYTNTAYYTNATHGARMGNAARTAYWSNCCNTGYGCNTGGGARGTNGTNMGNGCNGARATHATGMGNWSNYTNWSNTTYWSNACNAAYYTNCARAARMGNYTNMGNMGNAARGAY

SEQ ID NO: 4 - protein, 189 aa, Homo sapiens
MALSFSLLMAVLVLSYKSICSLGCDLPQTHSLGNRRALILLGQMGRISPFSCLKDRHDFRIPQEEFDGNQFQKAQAISVLHEMIQQTFNLFSTEDSSAAWEQSLLEKFSTELYQQLNDLEACVIQEVGVEETPLMNEDSILAVRKYFQRITLYLIERKYSPCAWEVVRAEIMRSLSFSTNLQKRLRRKD

SEQ ID NO: 5 - protein, 189 aa, Homo sapiens
MALPFALMMALVVLSCKSSCSLGCNLSQTHSLNNRRTLMLMAQMRRISPFSCLKDRHDFEFPQEEFDGNQFQKAQAISVLHEMMQQTFNLFSTKNSSAAWDETLLEKFYIELFQQMNDLEACVIQEVGVEETPLMNEDSILAVKKYFQRITLYLMEKKYSPCAWEVVRAEIMRSLSFSTNLQKRLRRKD